European Patent Application EP 4 722 241 A1, published April 8, 2026. Title: anti-synaptotagmin-2 antibody. Applicant: Jiksak Bioengineering, Inc. The sequence listing filed with the application follows.

SEQUENCE LISTING (21 sequences)

SEQ ID NO: 1 - protein, 118 aa, synthetic construct
EVQLQESGAELVRPGASVKLSCKASGYTFTDYEMHWVKQTPVHGLEWIGAIDPETGGTAYNQKFKGKATLTADKSSSTAYMELRSLTSEDSAVYYCTRGNDGYNEDYWGQGTTLTVSS

SEQ ID NO: 2 - protein, 112 aa, synthetic construct
DVLMTQTPLTLSVTIGQPASISCKSSQSLLDSDGKTYLNWLLQRPGQSPKRLIYLVSKLDSGVPDRFTGSGSGTDFTLKISRVEAEDLGVYYCWQDTHFPYTFGGGTKLEIK

SEQ ID NO: 3 - protein, 5 aa, synthetic construct
DYEMH

SEQ ID NO: 4 - protein, 17 aa, synthetic construct
AIDPETGGTAYNQKFKG

SEQ ID NO: 5 - protein, 9 aa, synthetic construct
GNDGYNEDY

SEQ ID NO: 6 - protein, 16 aa, synthetic construct
KSSQSLLDSDGKTYLN

SEQ ID NO: 7 - protein, 7 aa, synthetic construct
LVSKLDS

SEQ ID NO: 8 - protein, 9 aa, synthetic construct
WQDTHFPYT

SEQ ID NO: 9 - protein, 419 aa, Homo sapiens
MRNIFKRNQEPIVAPATTTATMPIGPVDNSTESGGAGESQEDMFAKLKEKLFNEINKIPLPPWALIAIAVVAGLLLLTCCFCICKKCCCKKKKNKKEKGKGMKNAMNMKDMKGGQDDDDAETGLTEGEGEGEEEKEPENLGKLQFSLDYDFQANQLTVGVLQAAELPALDMGGTSDPYVKVFLLPDKKKKYETKVHRKTLNPAFNETFTFKVPYQELGGKTLVMAIYDFDRFSKHDIIGEVKVPMNTVDLGQPIEEWRDLQGGEKEEPEKLGDICTSLRYVPTAGKLTVCILEAKNLKKMDVGGLSDPYVKIHLMQNGKRLKKKKTTVKKKTLNPYFNESFSFEIPFEQIQKVQVVVTVLDYDKLGKNEAIGKIFVGSNATGTELRHWSDMLANPRRPIAQWHSLKPEEEVDALLGKNK

SEQ ID NO: 10 - protein, 422 aa, Mus musculus
MRNIFKRNQEPNVAPATTTATMPLAPVAPADNSTESTGPGESQEDMFAKLKEKFFNEINKIPLPPWALIAMAVVAGLLLLTCCFCICKKCCCKKKKNKKEKGKGMKNAMNMKDMKGGQDDDDAETGLTEGEGEGEEEKEPENLGKLQFSLDYDFQANQLTVGVLQAAELPALDMGGTSDPYVKVFLLPDKKKKYETKVHRKTLNPAFNETFTFKVPYQELAGKTLVMAIYDFDRFSKHDIIGEVKVPMNTVDLGQPIEEWRDLQGGEKEEPEKLGDICTSLRYVPTAGKLTVCILEAKNLKKMDVGGLSDPYVKIHLMQNGKRLKKKKTTVKKKTLNPYFNESFSFEIPFEQIQKVQVVVTVLDYDKLGKNEAIGKIFVGSNATGTELRHWSDMLANPRRPIAQWHSLKPEEEVDALLGKNK

SEQ ID NO: 11 - protein, 62 aa, Homo sapiens
MRNIFKRNQEPIVAPATTTATMPIGPVDNSTESGGAGESQEDMFAKLKEKLFNEINKIPLPP

SEQ ID NO: 12 - protein, 60 aa, Mus musculus
MRNIFKRNQEPNVAPATTTATMPLAPVAPADNSTESTGPGESQEDMFAKLKEKFFNEINK

SEQ ID NO: 13 - protein, 63 aa, synthetic construct
  SITE 63: note = an additional Cysteine residue for binding to the carrier protein
MRNIFKRNQEPIVAPATTTATMPIGPVDNSTESGGAGESQEDMFAKLKEKLFNEINKIPLPPC

SEQ ID NO: 14 - protein, 63 aa, synthetic construct
  SITE 63: note = an additional Lysine residue bound to biotin
MRNIFKRNQEPIVAPATTTATMPIGPVDNSTESGGAGESQEDMFAKLKEKLFNEINKIPLPPK

SEQ ID NO: 15 - protein, 66 aa, synthetic construct
  SITE 66: note = an additional Lysine residue bound to biotin
MRNIFKRNQEPNVAPATTTATMPLAPVAPADNSTESTGPGESQEDMFAKLKEKFFNEINKIPLPPK

SEQ ID NO: 16 - protein, 59 aa, synthetic construct
  SITE 59: note = an additional Lysine residue bound to biotin
MVSESHHEALAAPPVTTVATVLPSNATEPASPGEGKEDAFSKLKEKFMNELHKIPLPPK

SEQ ID NO: 17 - protein, 118 aa, synthetic construct
QVQLQQSGAELVRPGASVKLSCKASGYTFTDYEMHWVKQTPVHGLEWIGAIDPETGGTAYNQKFKGKATLTADKSSSTAYMELRSLTSEDSAVYYCTRGNDGYNEDYWGQGTSLTVSS

SEQ ID NO: 18 - protein, 112 aa, synthetic construct
DIVMTQSPLTLSVTIGQPASISCKSSQSLLDSDGKTYLNWLLQRPGQSPKRLIYLVSKLDSGVPDRFTGSGSGTDFTLKISRVEAEDLGVYYCWQDTHFPYTFGGGTKLEIK

SEQ ID NO: 19 - DNA, 8353 bp, synthetic construct
  misc_feature 1028..1090: note = Leader sequence
  misc_feature 1091..2347: note = human SYT2 sequence
  source 1..8353: mol_type = other DNA
aacaaaatattaacgcttacaatttccattcgccattcaggctgcgcaactgttgggaagggcgatcggtgcgggcctcttcgctattacgccagctggcgaaagggggatgtgctgcaaggcgattaagttgggtaacgccagggttttcccagtcacgacgttgtaaaacgacggccagtgccaagctgatctatacattgaatcaatattggcaattagccatattagtcattggttatatagcataaatcaatattggctattggccattgcatacgttgtatctatatcataatatgtacatttatattggctcatgtccaatatgaccgccatgttgacattgattattgactagttattaatagtaatcaattacggggtcattagttcatagcccatatatggagttccgcgttacataacttacggtaaatggcccgcctggctgaccgcccaacgacccccgcccattgacgtcaataatgacgtatgttcccatagtaacgccaatagggactttccattgacgtcaatgggtggagtatttacggtaaactgcccacttggcagtacatcaagtgtatcatatgccaagtccgccccctattgacgtcaatgacggtaaatggcccgcctggcattatgcccagtacatgaccttacgggactttcctacttggcagtacatctacgtattagtcatcgctattaccatggtgatgcggttttggcagtacaccaatgggcgtggatagcggtttgactcacggggatttccaagtctccaccccattgacgtcaatgggagtttgttttggcaccaaaatcaacgggactttccaaaatgtcgtaataaccccgccccgttgacgcaaatgggcggtaggcgtgtacggtgggaggtctatataagcagagctcgtttagtgaaccgtcagaattttgtaatacgactcactatagggcggccgggaattcgtcgactggatccggtaccgaggagatctgccgccgcgatcgcatggagacagacacactcctgctatgggtactgctgctctgggttccaggttccactggtgacatgaggaacattttcaagaggaaccaggagcctattgtggctcctgccaccaccaccgccacgatgcccattggacccgtggacaactccactgagagtgggggtgctggggagagccaggaggacatgtttgccaaactgaaggagaagttattcaatgagataaacaagattcccttaccaccctgggcactgatcgccattgctgtggttgctgggctcctgcttctcacctgctgcttctgcatctgcaagaaatgctgctgcaagaagaagaagaacaagaaggagaagggcaaaggcatgaagaatgccatgaacatgaaggacatgaaagggggtcaggatgacgacgacgcagagacaggcctgactgagggggaaggtgaaggggaggaggagaaagagccagagaacctgggcaaactgcagttttccctggactatgattttcaggctaatcagcttactgtgggcgttctgcaggctgctgaactgcctgccctggacatgggaggcacctcagacccttatgtcaaggtcttcctccttcctgacaagaagaagaaatatgagaccaaagtccatcggaagacactgaaccctgccttcaatgaaaccttcaccttcaaggtgccataccaggagcttgggggcaaaactctggtgatggccatctatgactttgaccgcttctccaaacatgacatcattggagaggtaaaggtgcctatgaacacagtggacctcggccagcccattgaggagtggagagacctgcaaggcggggaaaaggaggagccggagaagctgggcgacatctgcacctccctgcgctatgtgcccacggccgggaagctcactgtctgcatcctggaggctaagaacctcaagaagatggacgtgggcggcctttcagacccgtacgtgaagatccacctgatgcagaatggcaagaggctcaagaagaagaagacaaccgtgaagaagaagaccctgaacccatacttcaacgagtccttcagctttgagatccccttcgagcagattcagaaagtccaggtagtggtcaccgtgctggactatgacaagctgggcaagaacgaagccataggcaagatcttcgtgggcagcaatgccacgggcacagagctgcggcactggtccgacatgctggccaacccccggaggcccatcgcccagtggcactcgctcaagcctgaggaggaggtggatgcactcctgggcaagaacaagacgcgtacgcggccgctcgagcagaaactcatctcagaagaggatctggcagcaaatgatatcctggattacaaggatgacgacgataaggtttaaacgtagcggccgcaaattccgcccctctccctcccccccccctaacgttactggccgaagccgcttggaataaggccggtgtgcgtttgtctatatgttattttccaccatattgccgtcttttggcaatgtgagggcccggaaacctggccctgtcttcttgacgagcattcctaggggtctttcccctctcgccaaaggaatgcaaggtctgttgaatgtcgtgaaggaagcagttcctctggaagcttcttgaagacaaacaacgtctgtagcgaccctttgcaggcagcggaaccccccacctggcgacaggtgcctctgcggccaaaagccacgtgtataagatacacctgcaaaggcggcacaaccccagtgccacgttgtgagttggatagttgtggaaagagtcaaatggctctcctcaagcgtattcaacaaggggctgaaggatgcccagaaggtaccccattgtatgggatctgatctggggcctcggtgcacatgctttacatgtgtttagtcgaggttaaaaaaacgtctaggccccccgaaccacggggacgtggttttcctttgaaaaacacgatgataatatggccacaaccatggagagcgacgagagcggcctgcccgccatggagatcgagtgccgcatcaccggcaccctgaacggcgtggagttcgagctggtgggcggcggagagggcacccccgagcagggccgcatgaccaacaagatgaagagcaccaaaggcgccctgaccttcagcccctacctgctgagccacgtgatgggctacggcttctaccacttcggcacctaccccagcggctacgagaaccccttcctgcacgccatcaacaacggcggctacaccaacacccgcatcgagaagtacgaggacggcggcgtgctgcacgtgagcttcagctaccgctacgaggccggccgcgtgatcggcgacttcaaggtgatgggcaccggcttccccgaggacagcgtgatcttcaccgacaagatcatccgcagcaacgccaccgtggagcacctgcaccccatgggcgataacgatctggatggcagcttcacccgcaccttcagcctgcgcgacggcggctactacagctccgtggtggacagccacatgcacttcaagagcgccatccaccccagcatcctgcagaacgggggccccatgttcgccttccgccgcgtggaggaggatcacagcaacaccgagctgggcatcgtggagtaccagcacgccttcaagaccccggatgcagatgccggtgaagaataatagccgctcatagctgtttcctgaacagatcccgggtggcatccctgtgacccctccccagtgcctctcctggccctggaagttgccactccagtgcccaccagccttgtcctaataaaattaagttgcatcattttgtctgactaggtgtccttctataatattatggggtggaggggggtggtatggagcaaggggcaagttgggaagacaacctgtagggcctgcggggtctattgggaaccaagctggagtgcagtggcacaatcttggctcactgcaatctccgcctcctgggttcaagcgattctcctgcctcagcctcccgagttgttgggattccaggcatgcatgaccaggctcagctaatttttgtttttttggtagagacggggtttcaccatattggccaggctggtctccaactcctaatctcaggtgatctacccaccttggcctcccaaattgctgggattacaggcgtgaaccactgctcccttccctgtccttctgattttaaaataactataccagcaggaggacgtccagacacagcataggctacctggccatgcccaaccggtgggacatttgagttgcttgcttggcactgtcctctcatgcgttgggtccactcagtagatgcctgttgaattgggtacgcggccagcttggctgtggaatgtgtgtcagttagggtgtggaaagtccccaggctccccagcaggcagaagtatgcaaagcatgcatctcaattagtcagcaaccaggtgtggaaagtccccaggctccccagcaggcagaagtatgcaaagcatgcatctcaattagtcagcaaccatagtcccgcccctaactccgcccatcccgcccctaactccgcccagttccgcccattctccgccccatggctgactaattttttttatttatgcagaggccgaggccgcctcggcctctgagctattccagaagtagtgaggaggcttttttggaggcctaggcttttgcaaaaagctcccgggagcttgtatatccattttcggatctgatcaagagacacgtacgaccatgaccgagtacaagcccacggtgcgcctcgccacccgcgacgacgtccccagggccgtacgcaccctcgccgccgcgttcgccgactaccccgccacgcgccacaccgtcgatccggaccgccacatcgagcgggtcaccgagctgcaagaactcttcctcacgcgcgtcgggctcgacatcggcaaggtgtgggtcgcggacgacggcgccgcggtggcggtctggaccacgccggagagcgtcgaagcgggggcggtgttcgccgagatcggcccgcgcatggccgagttgagcggttcccggctggccgcgcagcaacagatggaaggcctcctggcgccgcaccggcccaaggagcccgcgtggttcctggccaccgtcggcgtctcgcccgaccaccagggcaagggtctgggcagcgccgtcgtgctccccggagtggaggcggccgagcgcgccggggtgcccgccttcctggagacctccgcgccccgcaacctccccttctacgagcggctcggcttcaccgtcaccgccgacgtcgaggtgcccgaaggaccgcgcacctggtgcatgacccgcaagcccggtgcctgactgcagtgggactctggggttcgaaatgaccgaccaagcgacgcccaacctgccatcacgagatttcgattccaccgccgccttctatgaaaggttgggcttcggaatcgttttccgggacgccggctggatgatcctccagcgcggggatctcatgctggagttcttcgcccaccccaacttgtttattgcagcttataatggttacaaataaagcaatagcatcacaaatttcacaaataaagcatttttttcactgcattctagttgtggtttgtccaaactcatcaatgtatcttatcatgtctgtataccgtcgacctctagctagagcttggcgtaatcatggtcatagctgtttcctgtgtgaaattgttatccgctcacaattccacacaacatacgagccggaagcataaagtgtaaagcctggggtgcctaatgagtgagctaactcacattaattgcgttgcgctcactgcccgctttccagtcgggaaacctgtcgtgccagctgcattaatgaatcggccaacgcgcggggagaggcggtttgcgtattgggcgctcttccgcttcctcgctcactgactcgctgcgctcggtcgttcggctgcggcgagcggtatcagctcactcaaaggcggtaatacggttatccacagaatcaggggataacgcaggaaagaacatgtgagcaaaaggccagcaaaaggccaggaaccgtaaaaaggccgcgttgctggcgtttttccataggctccgcccccctgacgagcatcacaaaaatcgacgctcaagtcagaggtggcgaaacccgacaggactataaagataccaggcgtttccccctggaagctccctcgtgcgctctcctgttccgaccctgccgcttaccggatacctgtccgcctttctcccttcgggaagcgtggcgctttctcatagctcacgctgtaggtatctcagttcggtgtaggtcgttcgctccaagctgggctgtgtgcacgaaccccccgttcagcccgaccgctgcgccttatccggtaactatcgtcttgagtccaacccggtaagacacgacttatcgccactggcagcagccactggtaacaggattagcagagcgaggtatgtaggcggtgctacagagttcttgaagtggtggcctaactacggctacactagaagaacagtatttggtatctgcgctctgctgaagccagttaccttcggaaaaagagttggtagctcttgatccggcaaacaaaccaccgctggtagcggtggtttttttgtttgcaagcagcagattacgcgcagaaaaaaaggatctcaagaagatcctttgatcttttctacggggtctgacgctcagtggaacgaaaactcacgttaagggattttggtcatgagattatcaaaaaggatcttcacctagatccttttaaattaaaaatgaagttttaaatcaatctaaagtatatatgagtaaacttggtctgacagttaccaatgcttaatcagtgaggcacctatctcagcgatctgtctatttcgttcatccatagttgcctgactccccgtcgtgtagataactacgatacgggagggcttaccatctggccccagtgctgcaatgataccgcgagacccacgctcaccggctccagatttatcagcaataaaccagccagccggaagggccgagcgcagaagtggtcctgcaactttatccgcctccatccagtctattaattgttgccgggaagctagagtaagtagttcgccagttaatagtttgcgcaacgttgttgccattgctacaggcatcgtggtgtcacgctcgtcgtttggtatggcttcattcagctccggttcccaacgatcaaggcgagttacatgatcccccatgttgtgcaaaaaagcggttagctccttcggtcctccgatcgttgtcagaagtaagttggccgcagtgttatcactcatggttatggcagcactgcataattctcttactgtcatgccatccgtaagatgcttttctgtgactggtgagtactcaaccaagtcattctgagaatagtgtatgcggcgaccgagttgctcttgcccggcgtcaatacgggataataccgcgccacatagcagaactttaaaagtgctcatcattggaaaacgttcttcggggcgaaaactctcaaggatcttaccgctgttgagatccagttcgatgtaacccactcgtgcacccaactgatcttcagcatcttttactttcaccagcgtttctgggtgagcaaaaacaggaaggcaaaatgccgcaaaaaagggaataagggcgacacggaaatgttgaatactcatactcttcctttttcaatattattgaagcatttatcagggttattgtctcatgagcggatacatatttgaatgtatttagaaaaataaacaaataggggttccgcgcacatttccccgaaaagtgccacctgacgcgccctgtagcggcgcattaagcgcggcgggtgtggtggttacgcgcagcgtgaccgctacacttgccagcgccctagcgcccgctcctttcgctttcttcccttcctttctcgccacgttcgccggctttccccgtcaagctctaaatcgggggctccctttagggttccgatttagtgctttacggcacctcgaccccaaaaaacttgattagggtgatggttcacgtagtgggccatcgccctgatagacggtttttcgccctttgacgttggagtccacgttctttaatagtggactcttgttccaaactggaacaacactcaaccctatctcggtctattcttttgatttataagggattttgccgatttcggcctattggttaaaaaatgagctgatttaacaaaaatttaacgcgaatttt

SEQ ID NO: 20 - DNA, 63 bp, synthetic construct
  misc_feature 1..63: note = Leader sequence
  source 1..63: mol_type = other DNA
atggagacagacacactcctgctatgggtactgctgctctgggttccaggttccactggtgac

SEQ ID NO: 21 - DNA, 1257 bp, synthetic construct
  misc_feature 1..1257: note = human SYT2 sequence
  source 1..1257: mol_type = other DNA
atgaggaacattttcaagaggaaccaggagcctattgtggctcctgccaccaccaccgccacgatgcccattggacccgtggacaactccactgagagtgggggtgctggggagagccaggaggacatgtttgccaaactgaaggagaagttattcaatgagataaacaagattcccttaccaccctgggcactgatcgccattgctgtggttgctgggctcctgcttctcacctgctgcttctgcatctgcaagaaatgctgctgcaagaagaagaagaacaagaaggagaagggcaaaggcatgaagaatgccatgaacatgaaggacatgaaagggggtcaggatgacgacgacgcagagacaggcctgactgagggggaaggtgaaggggaggaggagaaagagccagagaacctgggcaaactgcagttttccctggactatgattttcaggctaatcagcttactgtgggcgttctgcaggctgctgaactgcctgccctggacatgggaggcacctcagacccttatgtcaaggtcttcctccttcctgacaagaagaagaaatatgagaccaaagtccatcggaagacactgaaccctgccttcaatgaaaccttcaccttcaaggtgccataccaggagcttgggggcaaaactctggtgatggccatctatgactttgaccgcttctccaaacatgacatcattggagaggtaaaggtgcctatgaacacagtggacctcggccagcccattgaggagtggagagacctgcaaggcggggaaaaggaggagccggagaagctgggcgacatctgcacctccctgcgctatgtgcccacggccgggaagctcactgtctgcatcctggaggctaagaacctcaagaagatggacgtgggcggcctttcagacccgtacgtgaagatccacctgatgcagaatggcaagaggctcaagaagaagaagacaaccgtgaagaagaagaccctgaacccatacttcaacgagtccttcagctttgagatccccttcgagcagattcagaaagtccaggtagtggtcaccgtgctggactatgacaagctgggcaagaacgaagccataggcaagatcttcgtgggcagcaatgccacgggcacagagctgcggcactggtccgacatgctggccaacccccggaggcccatcgcccagtggcactcgctcaagcctgaggaggaggtggatgcactcctgggcaagaacaag